European Patent Application EP 4 610 274 A1, published September 3, 2025. Title: Novel BBD29_RS14450 variant and a method for producing L-arginine using the same. Applicant: CJ CheilJedang Corporation. The sequence listing filed with the application follows.

SEQUENCE LISTING (100 sequences)

SEQ ID NO: 1 - protein, 121 aa, synthetic construct
VTAPLYKQIASLIEDSIVDGTLSIDQRVPSTNELAAFHRINPATALNGPTLLVEAGILYKKRGIGMFVSAQAPALIRERRDAAFAATYVAPLIDESIHLGFTRARIHALLDQVAESRGLYK

SEQ ID NO: 2 - DNA, 366 bp, synthetic construct
  source 1..366: mol_type = other DNA
gtgaccgcgcctctgtataaacagatcgcttctttgattgaggactccatcgttgacggaaccttgagcattgatcaacgcgtgccttctactaatgaactagccgcgttccatcgcattaatcccgccaccgcactcaacggcccgaccctccttgtcgaagccggcatcctctataagaagcgtggcattggcatgttcgtcagcgcccaggccccagcactcatccgagagcggcgagatgccgccttcgcagctacttatgtagcaccgcttatcgacgaatccatccaccttggtttcactcgtgcgcgcattcacgcccttttagaccaggtcgctgaaagtaggggcctgtacaagtag

SEQ ID NO: 3 - protein, 121 aa, synthetic construct
VTAPLYKQIASLIEDSIVDGTLSIDQRVPSTNELAAFHRINPATALNGLTLLVEAGILYKKRGIGMFVSAQAPALIRERRDAAFAATYVAPLIDESIHLGFTRARIHALLDQVAESRGLYK

SEQ ID NO: 4 - DNA, 366 bp, synthetic construct
  source 1..366: mol_type = other DNA
gtgaccgcgcctctgtataaacagatcgcttctttgattgaggactccatcgttgacggaaccttgagcattgatcaacgcgtgccttctactaatgaactagccgcgttccatcgcattaatcccgccaccgcactcaacggcctgaccctccttgtcgaagccggcatcctctataagaagcgtggcattggcatgttcgtcagcgcccaggccccagcactcatccgagagcggcgagatgccgccttcgcagctacttatgtagcaccgcttatcgacgaatccatccaccttggtttcactcgtgcgcgcattcacgcccttttagaccaggtcgctgaaagtaggggcctgtacaagtag

SEQ ID NO: 5 - protein, 495 aa, synthetic construct
MGESVSTDRYIPQQRTRYRQLLMEDLEIFDRHLQHSDFEDQGSIGLELELNLVDKHMQPALAGHAVLSHLDDEYQSEIGNFNVEMNHPPLSVKGDALRRLEQGITSRLGRVRAAATSENVNVAMIGTLPTITPEFLEDPAWMTQENRYRALSNAVMESRGELVHINIADREQIIHDFTDLAPESTCTSIQLHLQLAPNKFAAAWNASQAIAGVQAALSANSPLFLGRRVWHESRIPVFQQAIDTRTPELVNQGVRPRVWFGERWITSVFDLFEENVRYFSPLIAESRALSGTPMMKGKSPALHYLNLHNGTVWRWNRPIYSPGEERSHLRLENRLLPAGPTPIDITADAAFYYGLVKYLAEENRPVWSRLLFPDAEKNFQSGARSGLFARMTWPTLGQVNVANLVQEHLIPQARIGLERLEVNKDLIDQYLGIITERAKSRQNGATWQLRSLNKLEAHGSMPGSDARKAGLAAMLQQYLQNQESGQPVHTWSIGN

SEQ ID NO: 6 - DNA, 1488 bp, synthetic construct
  source 1..1488: mol_type = other DNA
atgggcgaatcagtaagtactgacaggtacattccgcagcagcgcacgcgttatcgccagctgctcatggaagatcttgagatttttgatcggcatttgcagcattccgattttgaggatcagggttccatcggcctcgagttggaactcaacctcgtggataagcatatgcaacctgctttggcaggccacgcggtgctttcccatttagacgatgagtaccagtcggagatcggtaactttaatgttgaaatgaaccacccgccactatccgttaaaggcgatgctttacgacgcctcgagcaaggcatcacctcgcgtctaggtcgcgtgcgcgcggccgccacatcggagaatgtgaacgtggcgatgatcggcacgctgcccaccatcactccggaatttcttgaagatccggcatggatgacccaagaaaaccgctaccgtgcgctgagcaatgcggtgatggaatcgcgtggcgagttagtgcacatcaacatcgccgaccgtgaacaaatcatccacgatttcactgatctcgcccccgaatcaacttgcacgtctattcagttgcacctgcaattagcgcccaataagtttgctgcagcgtggaatgcgtcgcaagcaatagctggtgttcaagcagctctttccgccaactccccacttttcctaggccgtcgggtgtggcatgaaagccgcattccagtgtttcaacaagccatcgatacgcgtactcctgaacttgtgaatcaaggagtccgccccagagtatggttcggcgaacgatggatcaccagtgtttttgatcttttcgaagaaaacgtacgctacttctcccctctcatcgcagaatcccgcgcactgtctggcacaccaatgatgaagggaaaatcccccgcactccactacctcaacctgcacaacggaacggtgtggcgctggaaccgacccatttactcaccgggcgaagagcgctcccacctgcgcctggaaaaccgtctcctacctgcaggtcccacccccatcgacatcactgccgatgccgctttctattacggtttggtcaaatatcttgccgaggaaaaccgccctgtctggtcacgtctcctattccctgatgcggaaaagaacttccaatccggtgcacgttcagggctgttcgcccgcatgacctggccaaccctcggacaagtcaacgttgcgaatctggtccaagagcacctcatccctcaagccagaatcggactggaacgacttgaagtaaataaagaccttatcgaccaatacctcggcatcatcaccgaacgcgcgaagtcccgccaaaacggtgccacctggcagttgcgtagcctcaacaagctggaagcacacggaagcatgccgggttccgatgctcgaaaagcaggtcttgcagcaatgttgcaacagtatttacagaatcaagaaagtggccaacctgtgcatacgtggagcatcggcaactaa

SEQ ID NO: 7 - protein, 495 aa, synthetic construct
MGESVSTDRYTPQQRTRYRQLLMEDLEIFDRHLQHSDFEDQGSIGLELELNLVDKHMQPALAGHAVLSHLDDEYQSEIGNFNVEMNHPPLSVKGDALRRLEQGITSRLGRVRAAATSENVNVAMIGTLPTITPEFLEDPAWMTQENRYRALSNAVMESRGELVHINIADREQIIHDFTDLAPESTCTSIQLHLQLAPNKFAAAWNASQAIAGVQAALSANSPLFLGRRVWHESRIPVFQQAIDTRTPELVNQGVRPRVWFGERWITSVFDLFEENVRYFSPLIAESRALSGTPMMKGKSPALHYLNLHNGTVWRWNRPIYSPGEERSHLRLENRLLPAGPTPIDITADAAFYYGLVKYLAEENRPVWSRLLFPDAEKNFQSGARSGLFARMTWPTLGQVNVANLVQEHLIPQARIGLERLEVNKDLIDQYLGIITERAKSRQNGATWQLRSLNKLEAHGSMPGSDARKAGLAAMLQQYLQNQESGQPVHTWSIGN

SEQ ID NO: 8 - DNA, 1488 bp, synthetic construct
  source 1..1488: mol_type = other DNA
atgggcgaatcagtaagtactgacaggtacactccgcagcagcgcacgcgttatcgccagctgctcatggaagatcttgagatttttgatcggcatttgcagcattccgattttgaggatcagggttccatcggcctcgagttggaactcaacctcgtggataagcatatgcaacctgctttggcaggccacgcggtgctttcccatttagacgatgagtaccagtcggagatcggtaactttaatgttgaaatgaaccacccgccactatccgttaaaggcgatgctttacgacgcctcgagcaaggcatcacctcgcgtctaggtcgcgtgcgcgcggccgccacatcggagaatgtgaacgtggcgatgatcggcacgctgcccaccatcactccggaatttcttgaagatccggcatggatgacccaagaaaaccgctaccgtgcgctgagcaatgcggtgatggaatcgcgtggcgagttagtgcacatcaacatcgccgaccgtgaacaaatcatccacgatttcactgatctcgcccccgaatcaacttgcacgtctattcagttgcacctgcaattagcgcccaataagtttgctgcagcgtggaatgcgtcgcaagcaatagctggtgttcaagcagctctttccgccaactccccacttttcctaggccgtcgggtgtggcatgaaagccgcattccagtgtttcaacaagccatcgatacgcgtactcctgaacttgtgaatcaaggagtccgccccagagtatggttcggcgaacgatggatcaccagtgtttttgatcttttcgaagaaaacgtacgctacttctcccctctcatcgcagaatcccgcgcactgtctggcacaccaatgatgaagggaaaatcccccgcactccactacctcaacctgcacaacggaacggtgtggcgctggaaccgacccatttactcaccgggcgaagagcgctcccacctgcgcctggaaaaccgtctcctacctgcaggtcccacccccatcgacatcactgccgatgccgctttctattacggtttggtcaaatatcttgccgaggaaaaccgccctgtctggtcacgtctcctattccctgatgcggaaaagaacttccaatccggtgcacgttcagggctgttcgcccgcatgacctggccaaccctcggacaagtcaacgttgcgaatctggtccaagagcacctcatccctcaagccagaatcggactggaacgacttgaagtaaataaagaccttatcgaccaatacctcggcatcatcaccgaacgcgcgaagtcccgccaaaacggtgccacctggcagttgcgtagcctcaacaagctggaagcacacggaagcatgccgggttccgatgctcgaaaagcaggtcttgcagcaatgttgcaacagtatttacagaatcaagaaagtggccaacctgtgcatacgtggagcatcggcaactaa

SEQ ID NO: 9 - protein, 339 aa, synthetic construct
MSTSSDYSHALIRRPRRLRANPAMRELVAETALRPADLILPMFFADGIAEAREISSMPGVYQHTEDSLLRAAHEALDAGVRCVDLFGVPVDAAKDFNGSEAWSETGVLNRALSSLRKEFGDDLLIMADTCLDEFTDHGHCGVVTEDRHGNAIVDNDATLPLYQQMAVAQARAGAHIVSPSGMMDGQIAAIRAALDEEGYQDVAIMAYSAKYASAFFGPFREAVGSSLQGDRRTYQQDPANLRESLLEAELDIAEGADFIMVKPALPYLDVLTRIADTSPVPVAAYQVSGEYAMIQAAGRNGWVDLDAVMMESLTSIKRAGANQILTYFAVNAARALRNA

SEQ ID NO: 10 - DNA, 1020 bp, synthetic construct
  source 1..1020: mol_type = other DNA
atgagcacttcttctgattactcccacgcactaattcgtcgtccgcgccgacttcgcgccaaccctgcgatgcgggaactagtcgcggaaaccgcattgcgcccggcggatcttattttgcccatgttctttgcggatggaatcgccgaggcacgtgagatctcctccatgcctggcgtttatcagcacacggaagattcactgctgcgtgccgcccatgaggctttagatgcgggtgttcgttgcgttgatctgttcggtgttccagtggatgcggccaaggacttcaatggttccgaggcgtggtctgaaaccggtgtgttgaaccgtgcactttcatcgctgcgtaaggaattcggcgatgacctgctgattatggccgatacttgccttgatgagttcacggatcatggtcactgcggcgtcgttaccgaggaccgtcatggaaatgcaatcgtggacaacgatgccacgttgccgctgtaccagcagatggctgttgctcaggctcgtgccggtgcacatattgtgagcccttccggaatgatggacggccagatcgctgctattcgtgcagcgttggatgaggaaggctaccaggacgtcgccatcatggcgtattccgctaagtatgcttcagcgttctttggacctttccgcgaagcggtgggatcctccctccaaggcgatcgacgtacctaccagcaagatcctgcgaacctgcgtgaatcattgcttgaggcagaactagatatcgcagaaggcgcggacttcatcatggtcaaacctgcattgccctaccttgatgtgctgacccgcatcgctgatacctcacctgtcccagtggctgcctaccaagtttctggtgagtacgcgatgatccaagcagcaggccgcaacggttgggttgaccttgatgcagtgatgatggaatctttgacctccatcaagcgtgccggtgcaaaccaaatcctcacgtactttgccgttaacgctgcccgcgcgctgcgaaacgcttaa

SEQ ID NO: 11 - protein, 339 aa, synthetic construct
MSTSSDYSHALIRRPRRLRANPAMRELVAETALRPADLILPMFFADGIAEAREISSMPGVYQHTEDSLLRAAHEALDAGVRCVDLFGVPVDAAKDFNGSEAWSETGVLNRALSSLRKEFGDDLLIMADTCLDEFTDHGHCGVVTEDRHGNAIVDNDATLPLYQQMAVAQARAGAHIVSPSGMMDGQIAAIRAALDEEGYQDVAIMAYSAKYASAFFGPFREAVGSSLQGDRRTYQQDPANLRESLLEAELDIAEGADFIMVKPALPYLDVLTRIADTSPFPVAAYQVSGEYAMIQAAGRNGWVDLDAVMMESLTSIKRAGANQILTYFAVNAARALRNA

SEQ ID NO: 12 - DNA, 1020 bp, synthetic construct
  source 1..1020: mol_type = other DNA
atgagcacttcttctgattactcccacgcactaattcgtcgtccgcgccgacttcgcgccaaccctgcgatgcgggaactagtcgcggaaaccgcattgcgcccggcggatcttattttgcccatgttctttgcggatggaatcgccgaggcacgtgagatctcctccatgcctggcgtttatcagcacacggaagattcactgctgcgtgccgcccatgaggctttagatgcgggtgttcgttgcgttgatctgttcggtgttccagtggatgcggccaaggacttcaatggttccgaggcgtggtctgaaaccggtgtgttgaaccgtgcactttcatcgctgcgtaaggaattcggcgatgacctgctgattatggccgatacttgccttgatgagttcacggatcatggtcactgcggcgtcgttaccgaggaccgtcatggaaatgcaatcgtggacaacgatgccacgttgccgctgtaccagcagatggctgttgctcaggctcgtgccggtgcacatattgtgagcccttccggaatgatggacggccagatcgctgctattcgtgcagcgttggatgaggaaggctaccaggacgtcgccatcatggcgtattccgctaagtatgcttcagcgttctttggacctttccgcgaagcggtgggatcctccctccaaggcgatcgacgtacctaccagcaagatcctgcgaacctgcgtgaatcattgcttgaggcagaactagatatcgcagaaggcgcggacttcatcatggtcaaacctgcattgccctaccttgatgtgctgacccgcatcgctgatacctcacctttcccagtggctgcctaccaagtttctggtgagtacgcgatgatccaagcagcaggccgcaacggttgggttgaccttgatgcagtgatgatggaatctttgacctccatcaagcgtgccggtgcaaaccaaatcctcacgtactttgccgttaacgctgcccgcgcgctgcgaaacgcttaa

SEQ ID NO: 13 - protein, 138 aa, synthetic construct
MVIYRKLAASAAALALSASLVACGDSEDTTEETSTTSSSTTSSSSSSSSSSTAATSEESSAVEEPAVEAPVEEAPVEAPVEAPVEQAPVVEQAPVEQAPAPVQEAPAPVEQAPAPVQEAPAADAPPALPGGGGGHAGY

SEQ ID NO: 14 - DNA, 417 bp, synthetic construct
  source 1..417: mol_type = other DNA
atggttatttaccgtaagcttgcggcttccgctgcagcactggccctgtccgcatcactggtcgcttgtggcgactctgaggacaccaccgaagaaacctcaaccacctcttcttcgaccacttccagctcctccagcagctctagctccagcaccgcggctacttccgaggaatcttccgcagttgaagagccagcagtggaagctcctgtggaagaggctccagtcgaggctccagtcgaggcacctgttgagcaggcacctgtcgtggagcaagctccagttgagcaggctccggcaccggttcaggaagcacctgcaccagtcgagcaggctccggctccagttcaggaagcacctgcagctgacgcaccacctgcacttccaggtggtggcggcggacacgctggctactaa

SEQ ID NO: 15 - protein, 134 aa, synthetic construct
MVIYRKLAASAAALALSASLVACGDSEDTTEETSTTSSSTTSSSSSSSSSSTAATSEESSAVEEPAVEAPVEEAPVEAPVEQAPVVEQAPVEQAPAPVQEAPAPVEQAPAPVQEAPAADAPPALPGGGGGHAGY

SEQ ID NO: 16 - DNA, 405 bp, synthetic construct
  source 1..405: mol_type = other DNA
atggttatttaccgtaagcttgcggcttccgctgcagcactggccctgtccgcatcactggtcgcttgtggcgactctgaggacaccaccgaagaaacctcaaccacctcttcttcgaccacttccagctcctccagcagctctagctccagcaccgcggctacttctgaggaatcttccgcagttgaagagccagcagtggaagctcctgtggaagaggctccagtcgaggcacctgttgagcaggcacctgtcgtggagcaagctccagttgagcaggctccggcaccggttcaggaagcacctgcaccagtcgagcaggctccagctccagttcaggaagcacctgcagctgacgcgccacctgcacttccaggtggtggcggcggacacgctggctactaa

SEQ ID NO: 17 - protein, 138 aa, synthetic construct
MAIYRKLAASAAALALSASLVACGDSEDTTEETSTTSSSTTSSSSSSSSSSTAATSEESSAVEEPAVEAPVEEAPVEAPVEAPVEQAPVVEQAPVEQAPAPVQEAPAPVEQAPAPVQEAPAADAPPALPGGGGGHAGY

SEQ ID NO: 18 - DNA, 417 bp, synthetic construct
  source 1..417: mol_type = other DNA
atggctatttaccgtaagcttgcggcttccgctgcagcactggccctgtccgcatcactggtcgcttgtggcgactctgaggacaccaccgaagaaacctcaaccacctcttcttcgaccacttccagctcctccagcagctctagctccagcaccgcggctacttccgaggaatcttccgcagttgaagagccagcagtggaagctcctgtggaagaggctccagtcgaggctccagtcgaggcacctgttgagcaggcacctgtcgtggagcaagctccagttgagcaggctccggcaccggttcaggaagcacctgcaccagtcgagcaggctccggctccagttcaggaagcacctgcagctgacgcaccacctgcacttccaggtggtggcggcggacacgctggctactaa

SEQ ID NO: 19 - protein, 347 aa, synthetic construct
MIIKVAIAGASGYAGGEILRLLLGHPAYASGELEIGALTAASTAGSTLGELMPHIPQLADRVIQDTTAETLAGHDVVFLGLPHGFSAEIALQLGPDVTVIDCAADFRLQNAADWEKFYGSEHQGTWPYGIPEIPGHREALRGAKRVAVPGCFPTGATLALLPAVQAGLIEPDVSVVSITGVSGAGKKASVALLGSETMGSLKTYNTSGKHRHTPEIAQNLGEVSDKPVKVSFTPVLAPLPRGILTTATAPLKEGVTAEQARAVYEEFYAQETFVHVLPEGAQPQTQAVLGSNMCHVQVEIDEEAGKVLVTSAIDNLTKGTAGAAVQCMNLSVGFDEAAGLPQVGVAP

SEQ ID NO: 20 - DNA, 1044 bp, synthetic construct
  source 1..1044: mol_type = other DNA
atgataatcaaggttgcaatcgcaggagccagtggatatgccggcggagaaatccttcgtctccttttaggccatccagcttatgcatctggtgaactagaaatcggagcactcaccgcggcatcaaccgcaggcagcacgctcggtgaattgatgccacacattccgcagttggcggatcgtgttattcaagacaccacagctgaaactctagccggtcatgatgtcgtatttctaggacttccacacggattctctgcagaaattgcacttcagctcggaccagatgtcacagtgattgactgtgcagctgactttcgtctgcaaaatgctgcagattgggagaagttctacggctcagagcaccagggaacatggccttatggcattccagaaataccaggacaccgcgaggctcttcgtggtgctaagcgtgtagcagtgccaggatgtttcccaaccggtgcaaccttggctcttcttcctgcggttcaagcgggacttatcgagccagatgtttccgtagtgtccatcaccggcgtatcaggtgcaggtaagaaagcatctgttgcactacttggctcggaaaccatgggttcactcaagacgtacaacacctccggaaagcaccgccacaccccggaaattgcccagaacctcggcgaagtcagcgacaagccagtcaaggtgagcttcaccccagtgcttgcaccgttacctcgcggaattctcaccactgcaaccgcacctttgaaagaaggcgttaccgcagagcaggctcgcgcagtatatgaagagttctatgcacaggaaaccttcgtgcatgttcttccagaaggtgcacagccacaaacccaagcagttcttggctccaacatgtgccacgtgcaggtagaaattgatgaggaagcaggcaaagtccttgttacctccgcaatcgataacctcaccaagggaactgccggcgccgctgttcagtgcatgaacttaagcgttggctttgatgaggcagcaggcctgccacaggtcggcgtcgcaccttaa

SEQ ID NO: 21 - protein, 347 aa, synthetic construct
MTIKVAIAGASGYAGGEILRLLLGHPAYASGELEIGALTAASTAGSTLGELMPHIPQLADRVIQDTTAETLAGHDVVFLGLPHGFSAEIALQLGPDVTVIDCAADFRLQNAADWEKFYGSEHQGTWPYGIPEIPGHREALRGAKRVAVPGCFPTGATLALLPAVQAGLIEPDVSVVSITGVSGAGKKASVALLGSETMGSLKAYNTSGKHRHTPEIAQNLGEVSDKPVKVSFTPVLAPLPRGILTTATAPLKEGVTAEQARAVYEEFYAQETFVHVLPEGAQPQTQAVLGSNMCHVQVEIDEEAGKVLVTSAIDNLTKGTAGAAVQCMNLSVGFDEAAGLPQVGVAP

SEQ ID NO: 22 - DNA, 1044 bp, synthetic construct
  source 1..1044: mol_type = other DNA
atgacaatcaaggttgcaatcgcaggagccagtggatatgccggcggagaaatccttcgtctccttttaggccatccagcttatgcatctggtgaactagaaatcggagcactcaccgcggcatcaaccgcaggcagcacgctcggtgaattgatgccacacattccgcagttggcggatcgtgttattcaagacaccacagctgaaactctagccggtcatgatgtcgtatttctaggacttccacacggattctctgcagaaattgcacttcagctcggaccagatgtcacagtgattgactgtgcagctgactttcgtctgcaaaatgctgcagattgggagaagttctacggctcagagcaccagggaacatggccttatggcattccagaaataccaggacaccgcgaggctcttcgtggtgctaagcgtgtagcagtgccaggatgtttcccaaccggtgcaaccttggctcttcttcctgcggttcaagcgggacttatcgagccagatgtttccgtagtgtccatcaccggcgtatcaggtgcaggtaagaaagcatctgttgcactacttggctcggaaaccatgggttcactcaaggcgtacaacacctccggaaagcaccgccacaccccggaaattgcccagaacctcggcgaagtcagcgacaagccagtcaaggtgagcttcaccccagtgcttgcaccgttacctcgcggaattctcaccactgcaaccgcacctttgaaagaaggcgttaccgcagagcaggctcgcgcagtatatgaagagttctatgcacaggaaaccttcgtgcatgttcttccagaaggtgcacagccacaaacccaagcagttcttggctccaacatgtgccacgtgcaggtagaaattgatgaggaagcaggcaaagtccttgttacctccgcaatcgataacctcaccaagggaactgccggcgccgctgttcagtgcatgaacttaagcgttggctttgatgaggcagcaggcctgccacaggtcggcgtcgcaccttaa

SEQ ID NO: 23-44 - skipped (22 entries)

SEQ ID NO: 45 - DNA, 38 bp, synthetic construct
  source 1..38: mol_type = other DNA
tgaattcgagctcggtaccctgaggtacgcaaactttc

SEQ ID NO: 46 - DNA, 28 bp, synthetic construct
  source 1..28: mol_type = other DNA
ctgctgcggaatgtacctgtcagtactt

SEQ ID NO: 47 - DNA, 28 bp, synthetic construct
  source 1..28: mol_type = other DNA
gacaggtacattccgcagcagcgcacgc

SEQ ID NO: 48 - DNA, 38 bp, synthetic construct
  source 1..38: mol_type = other DNA
gtcgactctagaggatccccgaaatcgtggatgatttg

SEQ ID NO: 49 - DNA, 38 bp, synthetic construct
  source 1..38: mol_type = other DNA
tgaattcgagctcggtaccccatcgctgcgtaaggaat

SEQ ID NO: 50 - DNA, 28 bp, synthetic construct
  source 1..28: mol_type = other DNA
gccactgggacaggtgaggtatcagcga

SEQ ID NO: 51 - DNA, 28 bp, synthetic construct
  source 1..28: mol_type = other DNA
tacctcacctgtcccagtggctgcctac

SEQ ID NO: 52 - DNA, 38 bp, synthetic construct
  source 1..38: mol_type = other DNA
gtcgactctagaggatcccctgaagaatcccatgacca

SEQ ID NO: 53 - DNA, 38 bp, synthetic construct
  source 1..38: mol_type = other DNA
tgaattcgagctcggtacccccactggcgttcaagatg

SEQ ID NO: 54 - DNA, 28 bp, synthetic construct
  source 1..28: mol_type = other DNA
acggtaaataaccatatgttttccttcc

SEQ ID NO: 55 - DNA, 28 bp, synthetic construct
  source 1..28: mol_type = other DNA
aaacatatggttatttaccgtaagcttg

SEQ ID NO: 56 - DNA, 38 bp, synthetic construct
  source 1..38: mol_type = other DNA
gtcgactctagaggatcccctgctgccaaaattcacga

SEQ ID NO: 57 - DNA, 38 bp, synthetic construct; identical to SEQ ID NO: 53
  source 1..38: mol_type = other DNA

SEQ ID NO: 58 - DNA, 28 bp, synthetic construct
  source 1..28: mol_type = other DNA
gctcaacaggtgcctcgactggagcctc

SEQ ID NO: 59 - DNA, 28 bp, synthetic construct
  source 1..28: mol_type = other DNA
ccagtcgaggcacctgttgagcaggcac

SEQ ID NO: 60 - DNA, 38 bp, synthetic construct; identical to SEQ ID NO: 56
  source 1..38: mol_type = other DNA

SEQ ID NO: 61 - DNA, 38 bp, synthetic construct
  source 1..38: mol_type = other DNA
tgaattcgagctcggtacccgagcactcaccgcggcat

SEQ ID NO: 62 - DNA, 28 bp, synthetic construct
  source 1..28: mol_type = other DNA
gtgttgtacgtcttgagtgaacccatgg

SEQ ID NO: 63 - DNA, 28 bp, synthetic construct
  source 1..28: mol_type = other DNA
ttcactcaagacgtacaacacctccgga

SEQ ID NO: 64 - DNA, 38 bp, synthetic construct
  source 1..38: mol_type = other DNA
gtcgactctagaggatccccttagatatgtttgttgtg

SEQ ID NO: 65-76 - skipped (12 entries)

SEQ ID NO: 77 - DNA, 38 bp, synthetic construct
  source 1..38: mol_type = other DNA
tgaattcgagctcggtaccccgatttctaattgggcac

SEQ ID NO: 78 - DNA, 28 bp, synthetic construct
  source 1..28: mol_type = other DNA
aaggagggtcgggccgttgagtgcggtg

SEQ ID NO: 79 - DNA, 28 bp, synthetic construct
  source 1..28: mol_type = other DNA
ctcaacggcccgaccctccttgtcgaag

SEQ ID NO: 80 - DNA, 38 bp, synthetic construct
  source 1..38: mol_type = other DNA
gtcgactctagaggatccccatcaccttgctcggtgtc

SEQ ID NO: 81-92 - skipped (12 entries)

SEQ ID NO: 93 - DNA, 38 bp, synthetic construct
  source 1..38: mol_type = other DNA
tgaattcgagctcggtaccccaaggttctggtcacggg

SEQ ID NO: 94 - DNA, 28 bp, synthetic construct
  source 1..28: mol_type = other DNA
gctgacagcctgagagaataccggagat

SEQ ID NO: 95 - DNA, 28 bp, synthetic construct
  source 1..28: mol_type = other DNA
gtattctctcaggctgtcagctgtggaa

SEQ ID NO: 96 - DNA, 38 bp, synthetic construct
  source 1..38: mol_type = other DNA
gtcgactctagaggatcccctgacggggttgagccaag

SEQ ID NO: 97 - protein, 359 aa, synthetic construct
MTSFNKDLTLRDTAIEGLLILDFPVHGDNRGWFKENWQREKMTALGLPDFGPVQNNMSFNATAGTTRGLHAEPWDKFVSVGTGKVFGAWCDLREGSPTFGAVVTQEITPDVGVYVPRGVANGFQALEDNTLYTYLVNDHWSPNAHYANVNLDMIDWPLPITEISDKDKNHPALADASPLPSRKVLVTGARGQLGTALRAVFPTAEFVGREELDITGPLDRPWKQYSAIINAAAYTAVDKAEDEGRAAAWAINAQAVASLATVARENNLTLVHISSDYVFDGTANGEYTEDAPLSPLGVYGQTKAAGDIAASTAPRHYVVRTSWVIGDGNNFVRGWEVMPCRRRSPVFSQAVSCGSSMPR

SEQ ID NO: 98 - DNA, 1080 bp, synthetic construct
  source 1..1080: mol_type = other DNA
atgacctcattcaataaagacctcaccctgcgtgacaccgccatcgagggtctgctgattcttgatttccccgtccacggtgataaccgcggctggttcaaggagaactggcagcgggagaagatgaccgcgcttggtctgccggatttcgggccggtgcaaaacaatatgagcttcaacgcgactgccggcaccacccgtggtctgcacgccgagccctgggacaagttcgtctccgtgggcaccggcaaggtcttcggcgcgtggtgcgatctgcgtgagggatcacccacctttggtgcggtggtcacccaggaaatcaccccggatgtcggcgtctacgtcccgcgcggggtggccaacggtttccaggcgctcgaggacaacaccctttatacctacctggtcaatgatcactggtcacctaacgcgcactacgccaacgtcaacctcgacatgatcgactggcccctgccgatcaccgagatctccgacaaggacaaaaaccaccccgcgcttgccgacgcctcccccctgccctcccgcaaggttctggtcacgggcgcgcgcgggcagttgggcaccgccctgcgggcggtgttcccgacggccgaattcgtcggccgtgaggaactcgatatcacgggcccgctggatcgtccctggaagcagtactccgccatcatcaacgccgcggcctacacggcagtggataaggccgaagacgaaggtcgcgctgcagcctgggccatcaacgctcaggcggtggccagcctggccacggtggcccgggagaacaacctcaccctggtgcatatctcctccgactacgtcttcgacggcaccgccaatggtgagtacaccgaggatgcgccactatcccccttgggtgtctacggccagaccaaggccgccggtgatatcgcagcgtccaccgcacctcggcattatgtggtgcgcaccagctgggtcatcggcgatggcaacaacttcgtgcggggctgggaagttatgccgtgcaggcgacgatctccggtattctctcaggctgtcagctgtggaagcagtatgccgcgttga

SEQ ID NO: 99 - protein, 359 aa, synthetic construct
MTSFNKDLTLRDTAIEGLLILDFPVHGDNRGWFKENWQREKMTALGLPDFGPVQNNMSFNATAGTTRGLHAEPWDKFVSVGTGKVFGAWCDLREGSPTFGAVVTQEITPDVGVYVPRGVANGFQALEDNTLYTYLVNDHWSPNAHYANVNLDMIDWPLPITEISDKDKNHPALADASPLPSRKVLVTGARGQLGTALRAVFPTAEFVGREELDITGPLDRPWKQYSAIINAAAYTAVDKAEDEGRAAAWAINAQAVASLATVARENNLTLVHISSDYVFDGTANGEYTEDAPLSPLGVYGQTKAAGDIAASTAPRHYVVRTSWVIGDGNNFVRGWEVMPCRRRSPVFSRAVSCGSSMPR

SEQ ID NO: 100 - DNA, 1080 bp, synthetic construct
  source 1..1080: mol_type = other DNA
atgacctcattcaataaagacctcaccctgcgtgacaccgccatcgagggtctgctgattcttgatttccccgtccacggtgataaccgcggctggttcaaggagaactggcagcgggagaagatgaccgcgcttggtctgccggatttcgggccggtgcaaaacaatatgagcttcaacgcgactgccggcaccacccgtggtctgcacgccgagccctgggacaagttcgtctccgtgggcaccggcaaggtcttcggcgcgtggtgcgatctgcgtgagggatcacccacctttggtgcggtggtcacccaggaaatcaccccggatgtcggcgtctacgtcccgcgcggggtggccaacggtttccaggcgctcgaggacaacaccctttatacctacctggtcaatgatcactggtcacctaacgcgcactacgccaacgtcaacctcgacatgatcgactggcccctgccgatcaccgagatctccgacaaggacaaaaaccaccccgcgcttgccgacgcctcccccctgccctcccgcaaggttctggtcacgggcgcgcgcgggcagttgggcaccgccctgcgggcggtgttcccgacggccgaattcgtcggccgtgaggaactcgatatcacgggcccgctggatcgtccctggaagcagtactccgccatcatcaacgccgcggcctacacggcagtggataaggccgaagacgaaggtcgcgctgcagcctgggccatcaacgctcaggcggtggccagcctggccacggtggcccgggagaacaacctcaccctggtgcatatctcctccgactacgtcttcgacggcaccgccaatggtgagtacaccgaggatgcgccactatcccccttgggtgtctacggccagaccaaggccgccggtgatatcgcagcgtccaccgcacctcggcattatgtggtgcgcaccagctgggtcatcggcgatggcaacaacttcgtgcggggctgggaagttatgccgtgcaggcgacgatctccggtattctctcgggctgtcagctgtggaagcagtatgccgcgttga